European Patent Application EP 4 148 130 A1, published March 15, 2023. Title: Topogami and method for making interlocked single stranded DNA rings. Applicant: Uniwersytet Jagielloñski. The sequence listing filed with the application follows.

SEQUENCE LISTING (124 sequences)

SEQ ID NO: 1 - DNA, 2616 bp, artificial
  Large circle sequence
caaccgttcgaaatattataaattatcagacatagtaaaacggcttcgtttgagtgtccattaaatcgtcattttggcataatagacacatcgtgtctgatattcgatttaaggtacatttttatgcgaattctttatccgcttcatcaagatgaaaataacgcgccagctgcctcgcgcgtttcggtgatgacggtgaaaacctctgacacatgcagctcccggagacggtcacagcttgtctgtaagcggatgccgggagcagacaagcccgtcagggcgcgtcagcgggtgttggcgggtgtcggggcgcagccatgacccagtcacgtagcgatagcggagtgtatactggcttaactatgcggcatcagagcagattgtactgagagtgcaccatatgcggtgtgaaataccgcacagatgcgtaaggagaaaataccgcatcaggcgctcttccgcttcctcgctcactgactcgctgcgctcggtcgttcggctgcggcgagcggtatcagctcactcaaaggcggtaatacggttatccacagaatcaggggataacgcaggaaagaacatgtgagcaaaaggccagcaaaaggccaggaaccgtaaaaaggccgcgttgctggcgtttttccataggctccgcccccctgacgagcatcacaaaaatcgacgctcaagtcagaggtggcgaaacccgacaggactataaagataccaggcgtttccccctggaagctccctcgtgcgctctcctgttccgaccctgccgcttaccggatacctgtccgcctttctcccttcgggaagcgtggcgctttctcatagctcacgctgtaggtatctcagttcggtgtaggtcgttcgctccaagctgggctgtgtgcacgaaccccccgttcagcccgaccgctgcgccttatccggtaactatcgtcttgagtccaacccggtaagacacgacttatcgccactggcagcagccactggtaacaggattagcagagcgaggtatgtaggcggtgctacagagttcttgaagtggtggcctaactacggctacactagaaggacagtatttggtatctgcgctctgctgaagccagttaccttcggaaaaagagttggtagctcttgatccggcaaacaaaccaccgctggtagcggtggtttttttgtttgcaagcagcagattacgcgcagaaaaaaaggatctcaagaagatcctttgatcttttctacggggtctgacgctcagtggaacgaaaactcacgttaagggattttggtcatgagattatcaaaaaggatcttcacctagatccttttaaattaaaaatgaagttttaaatcaatctaaagtatatatgagtaaacttggtctgacagttaccaatgcttaatcagtgaggcacctatctcagcgatctgtctatttcgttcatccatagttgcctgactccccgtcgtgtagataactacgatacgggagggcttaccatctggccccagtgctgcaatgataccgcgagacccacgctcaccggctccagatttatcagcaataaaccagccagccggaagggccgagcgcagaagtggtcctgcaactttatccgcctccatccagtctattaattgttgccgggaagctagagtaagtagttcgccagttaatagtttgcgcaacgttgttgccattgctgcaggcatcgtggtgtcacgctcgtcgtttggtatggcttcattcagctccggttcccaacgatcaaggcgagttacatgatcccccatgttgtgcaaaaaagcggttagctccttcggtcctccgatcgttgtcagaagtaagttggccgcagtgttatcactcatggttatggcagcactgcataattctcttactgtcatgccatccgtaagatgcttttctgtgactggtgagtactcaaccaagtcattctgagaatagtgtatgcggcgaccgagttgctcttgcccggcgtcaacacgggataataccgcgccacatagcagaactttaaaagtgctcatcattggaaaacgttcttcggggcgaaaactctcaaggatcttaccgctgttgagatccagttcgatgtaacccactcgtgcacccaactgatcttcagcatcttttactttcaccagcgtttctgggtgagcaaaaacaggaaggcaaaatgccgcaaaaaagggaataagggcgacacggaaatgttgaatactcatactcttcctttttcaatattattgaagcatttatcagggttattgtctcatgagcggatacatatttgaatgtatttagaaaaataaacaaataggggttccgcgcacatttccccgaaaagtgccacctgacgtctaagaaaccattattatcatgacattaacctataaaaataggcgtatcacgaggccctttcgtcttcaagaattctttatccgcttcatcaagatgaaaataacgcgccagctgaagttcatcgggttcgccagtgaacctgccataactctcaacctgctcagtggtcaaaaaatcaacgggcatatcggcctccctgcctgacggcttttttaacacaactg

SEQ ID NO: 2 - DNA, 2315 bp, artificial
  Small circle sequence
cagttgtgttaaaaaagccgtcaggcagggaggccgatatgcccgttgattttttgaccactgagcaggttgagagttatggcaggttcactggcgaacccgatgaacttcagctgcggtaaagctcatcagcgtggtcgtgaagcgattcacagatgtctgcctgttcatccgcgtccagctcgttgagtttctccagaagcgttaatgtctggcttctgataaagcgggccatgttaagggcggttttttcctgtttggtcactgatgcctccgtgtaagggggatttctgttcatgggggtaatgataccgatgaaacgagagaggatgctcacgatacgggttactgatgatgaacatgcccggttactggaacgttgtgagggtaaacaactggcggtatggatgcggcgggaccagagaaaaatcactcagggtcaatgccagcgcttcgttaatacagatgtaggtgttccacagggtagccagcagcatcctgcgatgcagatccggaacataatggtgcagggcgctgacttccgcgtttccagactttacgaaacacggaaaccgaagaccattcatgttgttgctcaggtcgcagacgttttgcagcagcagtcgcttcacgttcgctcgcgtatcggtgattcattctgctaaccagtaaggcaaccccgccagcctagccgggtcctcaacgacaggagcacgatcatgcgcacccgtggccaggacccaacgctgcccgagatgcgccgcgtgcggctgctggagatggcggacgcgatggatatgttctgccaagggttggtttgcgcattcacagttctccgcaagaattgattggctccaattcttggagtggtgaatccgttagcgaggtgccgccggcttccattcaggtcgaggtggcccggctccatgcaccgcgacgcaacgcggggaggcagacaaggtatagggcggcgcctacaatccatgccaacccgttccatgtgctcgccgaggcggcataaatcgccgtgacgatcagcggtccagtgatcgaagttaggctggtaagagccgcgagcgatccttgaagctgtccctgatggtcgtcatctacctgcctggacagcatggcctgcaacgcgggcatcccgatgccgccggaagcgagaagaatcataatggggaaggccatccagcctcgcgtcgcgaacgccagcaagacgtagcccagcgcgtcggccgccatgccggcgataatggcctgcttctcgccgaaacgtttggtggcgggaccagtgacgaaggcttgagcgagggcgtgcaagattccgaataccgcaagcgacaggccgatcatcgtcgcgctccagcgaaagcggtcctcgccgaaaatgacccagagcgctgccggcacctgtcctacgagttgcatgataaagaagacagtcataagtgcggcgacgatagtcatgccccgcgcccaccggaaggagctgactgggttgaaggctctcaagggcatcggtcgacgctctcccttatgcgactcctgcattaggaagcagcccagtagtaggttgaggccgttgagcaccgccgccgcaaggaatggtgcatgcaaggagatggcgcccaacagtcccccggccacggggcctgccaccatacccacgccgaaacaagcgctcatgagcccgaagtggcgagcccgatcttccccatcggtgatgtcggcgatataggcgccagcaaccgcacctgtggcgccggtgatgccggccacgatgcgtccggcgtagaggatccacaggacgggtgtggtcgccatgatcgcgtagtcgatagtggctccaagtagcgaagcgagcaggactgggcggcggccaaagcggtcggacagtgctccgagaacgggtgcgcatagaaattgcatcaacgcatatagcgctagcagcacgccatagtgactggcgatgctgtcggaatggacgatatcccgcaagaggcccggcagtaccggcataaccaagcctatgcctacagcatccagggtgacggtgccgaggatgacgatgagcgcattgttagatttcatacacggtgcctgactgcgttagcaatttaactgtgataaactaccgcattaaagcttatcgatgataagctgtcaaagctcttcatgagaattcgcataaaaatgtaccttaaatcgaatatcagacacgatgtgtctattatgccaaaatgacgatttaatggacactcaaacgaagccgttttactatgtctgataatttataatatttcgaacggttg

SEQ ID NO: 3 - DNA, 28 bp, artificial
  001 0H108-1H110 Large
tatccgcttcatcgtaagcggatgtttt

SEQ ID NO: 4 - DNA, 28 bp, artificial
  002 1H56-0H39 Large
tctgacacgtttcggtgatgacggtttt

SEQ ID NO: 5 - DNA, 32 bp, artificial
  003 1H72-3H71 Large
cccggagacgtcagcgggtgttggtggcttaa

SEQ ID NO: 6 - DNA, 48 bp, artificial
  004 1H88-1H71 Large
gcttgtctaagatgaaaataacgcgccagctgcctcgcgcatgcagct

SEQ ID NO: 7 - DNA, 30 bp, artificial
  TTTTCCGGGAGCAGAACTGAGAGTGCTTTT
ttttccgggagcagaactgagagtgctttt

SEQ ID NO: 8 - DNA, 30 bp, artificial; identical to SEQ ID NO: 7
  006 3H33-4H33 Large

SEQ ID NO: 9 - DNA, 32 bp, artificial
  007 3H56-1H55 Large
gtgtataccgggtgtcggggcgcatgaaaacc

SEQ ID NO: 10 - DNA, 32 bp, artificial
  008 3H72-5H71 Large
ctatgcgggatgcgtaaggagaaacgttcggc

SEQ ID NO: 11 - DNA, 32 bp, artificial
  009 3H88-1H87 Large
cagattgtcaagcccgtcagggcgcggtcaca

SEQ ID NO: 12 - DNA, 30 bp, artificial
  010 4H110-5H110 Large
ttttaccatatgcggcaaaggcggtatttt

SEQ ID NO: 13 - DNA, 30 bp, artificial
  011 5H33-6H33 Large
ttttctcgctcactggcaaaaggccatttt

SEQ ID NO: 14 - DNA, 32 bp, artificial
  012 5H56-3H55 Large
cgctcggtataccgcatcaggcgcatagcgga

SEQ ID NO: 15 - DNA, 32 bp, artificial
  013 5H72-7H71 Large
tgcggcgaaacgcaggaaagaacacgtttttc

SEQ ID NO: 16 - DNA, 32 bp, artificial
  014 5H88-3H87 Large
agctcacttgtgaaataccgcacacatcagag

SEQ ID NO: 17 - DNA, 30 bp, artificial
  015 6H110-7H110 Large
ttttatacggttatccatcacaaaaatttt

SEQ ID NO: 18 - DNA, 32 bp, artificial
  017 7H56-5H55 Large
gttgctggtgtgagcaaaaggccaactcgctg

SEQ ID NO: 19 - DNA, 32 bp, artificial
  019 7H88-5H87 Large
ctgacgagcacagaatcaggggatgcggtatc

SEQ ID NO: 20 - DNA, 30 bp, artificial
  050 20H110-21H110 Large
ttttcagtgctgcaattgttgccgggtttt

SEQ ID NO: 21 - DNA, 30 bp, artificial
  051 21H33-22H33 Large
ttttggaagggccgaggcatcgtggttttt

SEQ ID NO: 22 - DNA, 32 bp, artificial
  053 21H72-23H71 Large
atccgcctatagtttgcgcaacgtattcagct

SEQ ID NO: 23 - DNA, 30 bp, artificial
  055 22H110-23H110 Large
ttttaagctagagtattacatgatcctttt

SEQ ID NO: 24 - DNA, 30 bp, artificial
  056 23H33-24H33 Large
ttttgtcacgctcgtgttggccgcagtttt

SEQ ID NO: 25 - DNA, 32 bp, artificial
  057 23H56-21H55 Large
atggcttctgttgccattgctgcagcgcagaa

SEQ ID NO: 26 - DNA, 32 bp, artificial
  058 23H72-25H71 Large
ccggttcctccttcggtcctccgatgcataat

SEQ ID NO: 27 - DNA, 32 bp, artificial
  059 23H88-21H87 Large
aaggcgagagtagttcgccagttaccatccag

SEQ ID NO: 28 - DNA, 30 bp, artificial
  060 24H110-25H110 Large
ttttcccatgttgtgagatgcttttctttt

SEQ ID NO: 29 - DNA, 30 bp, artificial
  061 25H33-26H33 Large
tttttgttatcactcgctcttgcccgtttt

SEQ ID NO: 30 - DNA, 32 bp, artificial
  062 25H56-23H55 Large
ggcagcactcgttgtcagaagtaacgtttggt

SEQ ID NO: 31 - DNA, 32 bp, artificial
  063 25H72-27H71 Large
tctcttacattctgagaatagtgtcatagcag

SEQ ID NO: 32 - DNA, 32 bp, artificial
  064 25H88-23H87 Large
catccgtacaaaaaagcggttagccaacgatc

SEQ ID NO: 33 - DNA, 30 bp, artificial
  065 26H110-27H110 Large
tttttgtgactggtgaaaacgttctttttt

SEQ ID NO: 34 - DNA, 30 bp, artificial
  066 27H33-28H33 Large
ttttgcgtcaacacgcgtgcacccaatttt

SEQ ID NO: 35 - DNA, 32 bp, artificial
  067 27H56-25H55 Large
ccgcgccaatgcggcgaccgagttatggttat

SEQ ID NO: 36 - DNA, 32 bp, artificial
  068 27H72-29H71 Large
aactttaacgctgttgagatccagcagcgttt

SEQ ID NO: 37 - DNA, 32 bp, artificial
  069 27H88-25H87 Large
atcattggagtactcaaccaagtctgtcatgc

SEQ ID NO: 38 - DNA, 30 bp, artificial
  070 28H110-29H110 Large
ttttcggggcgaaaaaaaatgccgcatttt

SEQ ID NO: 39 - DNA, 30 bp, artificial
  071 29H33-30H33 Large
ttttctgatcttcagttattgaagcatttt

SEQ ID NO: 40 - DNA, 32 bp, artificial
  072 29H56-27H55 Large
actttcacttcgatgtaacccactggataata

SEQ ID NO: 41 - DNA, 32 bp, artificial
  073 29H72-31H71 Large
ctgggtgatgttgaatactcatacgatacata

SEQ ID NO: 42 - DNA, 32 bp, artificial
  AGGAAGGCCTCTCAAGGATCTTACAAGTGCTC
aggaaggcctctcaaggatcttacaagtgctc

SEQ ID NO: 43 - DNA, 30 bp, artificial
  075 30H110-31H110 Large
ttttaaaaagggaatcaaataggggttttt

SEQ ID NO: 44 - DNA, 30 bp, artificial
  076 31H33-32H33 Large
tttttttatcagggtcattaacctattttt

SEQ ID NO: 45 - DNA, 32 bp, artificial
  077 31H56-29H55 Large
catgagcgtcttcctttttcaatacatctttt

SEQ ID NO: 46 - DNA, 48 bp, artificial
  078 31H72-33H87 Large
tttgaatgacctgacgtctaagaacgtcttcaagaattctttatccgc

SEQ ID NO: 47 - DNA, 32 bp, artificial
  079 31H88-29H87 Large
aaaataaaaagggcgacacggaaagcaaaaac

SEQ ID NO: 48 - DNA, 30 bp, artificial
  080 32H110-33H110 Large
tttttccgcgcacatgatgaaaataacgcg

SEQ ID NO: 49 - DNA, 23 bp, artificial
  081 33H33-33H55 Large
ttttaaaaataggcgtatcacga

SEQ ID NO: 50 - DNA, 32 bp, artificial
  082 33H56-31H55 Large
ggccctttaccattattatcatgatattgtct

SEQ ID NO: 51 - DNA, 32 bp, artificial
  083 33H88-31H87 Large
ttcatcaattccccgaaaagtgcctatttaga

SEQ ID NO: 52 - DNA, 30 bp, artificial
  084 1H145-0H145 Small
ttttcgcattgttagagctgtcaaacatga

SEQ ID NO: 53 - DNA, 32 bp, artificial
  085 1H168-3H167 Small
cacggtgcggtgacggtgccgaggtagcagca

SEQ ID NO: 54 - DNA, 48 bp, artificial
  086 1H184-1H167 Small
gttagcaaataaactaccgcattaaagcttatcgatgataatttcata

SEQ ID NO: 55 - DNA, 39 bp, artificial
  087 2H222-3H199 Small
ttttccggcagtaccggcataaccaagcctacggaatgg

SEQ ID NO: 56 - DNA, 30 bp, artificial
  088 3H145-2H145 Small
ttttgcatatagcgcatgacgatgagtttt

SEQ ID NO: 57 - DNA, 32 bp, artificial
  089 3H168-5H167 Small
cgccatagacgggtgcgcatagaaaggacggg

SEQ ID NO: 58 - DNA, 32 bp, artificial
  090 3H184-1H183 Small
gatgctgttgcctacagcatccagctgactgc

SEQ ID NO: 59 - DNA, 32 bp, artificial
  091 3H200-5H199 Small
acgatatcggcggccaaagcggtcgatagtgg

SEQ ID NO: 60 - DNA, 30 bp, artificial
  092 4H222-3H222 Small
ttttcaggactgggcccgcaagaggctttt

SEQ ID NO: 61 - DNA, 30 bp, artificial
  093 5H145-4H145 Small
ttttagaggatccacattgcatcaactttt

SEQ ID NO: 62 - DNA, 32 bp, artificial
  094 5H168-7H167 Small
tgtggtcgtgatgccggccacgatccacgccg

SEQ ID NO: 63 - DNA, 32 bp, artificial
  GCGTAGTCGGACAGTGCTCCGAGATGACTGGC
gcgtagtcggacagtgctccgagatgactggc

SEQ ID NO: 64 - DNA, 32 bp, artificial
  096 5H200-7H199 Small
ctccaagtataggcgccagcaacctggcgagc

SEQ ID NO: 65 - DNA, 30 bp, artificial
  097 6H222-5H222 Small
ttttatgtcggcgatagcgaagcgagtttt

SEQ ID NO: 66 - DNA, 30 bp, artificial
  098 7H145-6H145 Small
tttttgccaccatacgcgtccggcgttttt

SEQ ID NO: 67 - DNA, 32 bp, artificial
  099 7H168-9H167 Small
aaacaagcgcccaacagtcccccgacgctctc

SEQ ID NO: 68 - DNA, 32 bp, artificial
  100 7H184-5H183 Small
gcccgaaggcacctgtggcgccggccatgatc

SEQ ID NO: 69 - DNA, 32 bp, artificial
  101 7H200-9H199 Small
ccgatcttgccgcaaggaatggtgagcagccc

SEQ ID NO: 70 - DNA, 30 bp, artificial
  102 8H222-7H222 Small
tttttgagcaccgccccccatcggtgtttt

SEQ ID NO: 71 - DNA, 30 bp, artificial
  103 9H145-8H145 Small
ttttggcatcggtcggccacggggcctttt

SEQ ID NO: 72 - DNA, 32 bp, artificial
  104 9H168-11H167 Small
ccttatgcgagctgactgggttgaaaaatgac

SEQ ID NO: 73 - DNA, 32 bp, artificial
  105 9H184-7H183 Small
cattaggacatgcaaggagatggcgctcatga

SEQ ID NO: 74 - DNA, 32 bp, artificial
  106 9H200-11H199 Small
agtagtagcgacgatagtcatgcctacgagtt

SEQ ID NO: 75 - DNA, 30 bp, artificial
  107 10H222-9H222 Small
ttttcataagtgcgggttgaggccgttttt

SEQ ID NO: 76 - DNA, 30 bp, artificial
  108 11H145-10H145 Small
ttttggtcctcgccgaggctctcaagtttt

SEQ ID NO: 77 - DNA, 32 bp, artificial
  109 11H168-13H167 Small
ccagagcgcgatcatcgtcgcgctcggcgata

SEQ ID NO: 78 - DNA, 32 bp, artificial
  110 11H184-9H183 Small
acctgtccccgcgcccaccggaaggactcctg

SEQ ID NO: 79 - DNA, 32 bp, artificial
  111 11H200-13H199 Small
gcatgatagtgcaagattccgaatttggtggc

SEQ ID NO: 80 - DNA, 30 bp, artificial
  112 12H222-11H222 Small
tttttgagcgagggcaagaagacagttttt

SEQ ID NO: 81 - DNA, 30 bp, artificial
  113 13H145-12H145 Small
ttttggccgccatgcccagcgaaagctttt

SEQ ID NO: 82 - DNA, 32 bp, artificial
  114 13H168-15H167 Small
atggcctgcgccagcaagacgtagatctacct

SEQ ID NO: 83 - DNA, 32 bp, artificial
  115 13H184-11H183 Small
cgaaacgtaccgcaagcgacaggcctgccggc

SEQ ID NO: 84 - DNA, 32 bp, artificial
  116 13H200-15H199 Small
gggaccagatggggaaggccatcccgggcatc

SEQ ID NO: 85 - DNA, 30 bp, artificial
  117 14H222-13H222 Small
ttttgaagaatcatatgacgaaggcttttt

SEQ ID NO: 86 - DNA, 30 bp, artificial
  118 15H145-14H145 Small
tttttgatggtcgtccccagcgcgtctttt

SEQ ID NO: 87 - DNA, 32 bp, artificial
  119 15H168-17H167 Small
gcctggacgccgcgagcgatccttgcggcgcc

SEQ ID NO: 88 - DNA, 32 bp, artificial
  120 15H184-13H183 Small
ctgcaacgagcctcgcgtcgcgaacttctcgc

SEQ ID NO: 89 - DNA, 30 bp, artificial
  122 16H222-15H222 Small
ttttcgtgacgatcagccggaagcgatttt

SEQ ID NO: 90 - DNA, 30 bp, artificial
  123 17H145-16H145 Small
ttttcaaggtatagggaagctgtccctttt

SEQ ID NO: 91 - DNA, 32 bp, artificial
  124 17H168-19H167 Small
tacaatcccaccgcgacgcaacgcacagttct

SEQ ID NO: 92 - DNA, 32 bp, artificial
  125 17H184-15H183 Small
ccgttccaagttaggctggtaagaagcatggc

SEQ ID NO: 93 - DNA, 32 bp, artificial
  126 17H200-19H199 Small
ccgaggcgttccattcaggtcgagtcttggag

SEQ ID NO: 94 - DNA, 30 bp, artificial
  127 18H222-17H222 Small
ttttgtgccgccggcgcataaatcgctttt

SEQ ID NO: 95 - DNA, 30 bp, artificial
  128 19H145-18H145 Small
tttttttgcgcattcggggaggcagatttt

SEQ ID NO: 96 - DNA, 32 bp, artificial
  129 19H168-21H167 Small
ccgcaagacgatggatatgttctgctagccgg

SEQ ID NO: 97 - DNA, 32 bp, artificial
  130 19H184-17H183 Small
gctccaatgtggcccggctccatgatgccaac

SEQ ID NO: 98 - DNA, 32 bp, artificial
  131 19H200-21H199 Small
tggtgaatgcgccgcgtgcggctgatgcgcac

SEQ ID NO: 99 - DNA, 30 bp, artificial
  132 20H222-19H222 Small
ttttctgcccgagatccgttagcgagtttt

SEQ ID NO: 100 - DNA, 30 bp, artificial
  133 21H145-20H145 Small
ttttaccccgccagcccaagggttggtttt

SEQ ID NO: 101 - DNA, 32 bp, artificial
  134 21H168-23H167 Small
gtcctcaatgattcattctgctaattccagac

SEQ ID NO: 102 - DNA, 32 bp, artificial
  135 21H184-19H183 Small
gcacgatcctggagatggcggacgattgattg

SEQ ID NO: 103 - DNA, 32 bp, artificial
  136 21H200-23H199 Small
ccgtggcccagcagtcgcttcacgccattcat

SEQ ID NO: 104 - DNA, 30 bp, artificial
  137 22H222-21H222 Small
ttttacgttttgcagaggacccaacgtttt

SEQ ID NO: 105 - DNA, 30 bp, artificial
  138 23H145-22H145 Small
ttttgacttccgcgtccagtaaggcatttt

SEQ ID NO: 106 - DNA, 32 bp, artificial
  139 23H168-25H167 Small
tttacgaaatccggaacataatggatgcggcg

SEQ ID NO: 107 - DNA, 32 bp, artificial
  140 23H184-21H183 Small
accgaagattcgctcgcgtatcggcgacagga

SEQ ID NO: 108 - DNA, 32 bp, artificial
  141 23H200-25H199 Small
gttgttgccacagggtagccagcatcaatgcc

SEQ ID NO: 109 - DNA, 30 bp, artificial
  142 24H222-23H222 Small
tttttgtaggtgttctcaggtcgcagtttt

SEQ ID NO: 110 - DNA, 30 bp, artificial
  143 25H145-24H145 Small
tttttggcggtatggtgcagggcgcttttt

SEQ ID NO: 111 - DNA, 32 bp, artificial
  144 25H168-27H167 Small
ggaccagatactggaacgttgtgaatgcctcc

SEQ ID NO: 112 - DNA, 32 bp, artificial
  145 25H184-23H183 Small
actcaggggcatcctgcgatgcagacacggaa

SEQ ID NO: 113 - DNA, 32 bp, artificial
  146 25H200-27H199 Small
agcgcttcgatacgggttactgatggggtaat

SEQ ID NO: 114 - DNA, 30 bp, artificial
  147 26H222-25H222 Small
ttttaggatgctcacgttaatacagatttt

SEQ ID NO: 115 - DNA, 30 bp, artificial
  148 27H145-26H145 Small
tttttttggtcactggggtaaacaactttt

SEQ ID NO: 116 - DNA, 32 bp, artificial
  149 27H168-29H167 Small
gtgtaaggggccatgttaagggcgatcagcgt

SEQ ID NO: 117 - DNA, 32 bp, artificial
  150 27H184-25H183 Small
tgttcatggatgaacatgcccggtgaaaaatc

SEQ ID NO: 118 - DNA, 32 bp, artificial
  151 27H200-29H199 Small
gataccgaagaagcgttaatgtctctgcctgt

SEQ ID NO: 119 - DNA, 30 bp, artificial
  152 28H222-27H222 Small
tttttgagtttctcctgaaacgagagtttt

SEQ ID NO: 120 - DNA, 30 bp, artificial
  153 29H145-28H145 Small
ttttcggtaaagctcgttttttcctgtttt

SEQ ID NO: 121 - DNA, 48 bp, artificial
  154 29H168-27H183 Small
ggtcgtgaagcgattcacagatgtggcttctgataaagcggggatttc

SEQ ID NO: 122 - DNA, 23 bp, artificial
  155 29H200-29H222 Small
tcatccgcgtccagctcgttttt

SEQ ID NO: 123 - DNA, 34 bp, artificial
  Nt.BspQI_rev
aattctcatgaagagctttgacagcttatcatcg

SEQ ID NO: 124 - DNA, 33 bp, artificial
  Nt.BspQI_for
gataagctgtcaaagctcttcatgagaattcgc